European Patent Application EP 4 524 258 A1, published March 19, 2025. Title: METHOD OF PURIFYING AND ANALYZING NUCLEIC ACID. Applicant: Gwangju Institute of Science and Technology. The sequence listing filed with the application follows.

SEQUENCE LISTING (12 sequences)

SEQ ID NO: 1 - skipped

SEQ ID NO: 2 - DNA, 27 bp, synthetic construct
  misc_feature 1..27: note = Synthetic Sequence
  source 1..27: mol_type = other DNA
tggtctcctccagtcaccaaatatgcg

SEQ ID NO: 3 - RNA, 58 nt, synthetic construct
  misc_feature 1..58: note = Synthetic Sequence
  source 1..58: mol_type = other RNA
tactcaacttgaaaaggtggcaccgattcggtgtttttcgcatatttggtgactggag

SEQ ID NO: 4 - RNA, 68 nt, synthetic construct
  misc_feature 1..68: note = Synthetic Sequence
  source 1..68: mol_type = other RNA
tttttttttttactcaacttgaaaaggtggctccgattcggtgtttttcgcatatttggtgactggag

SEQ ID NO: 5 - RNA, 58 nt, synthetic construct; identical to SEQ ID NO: 3
  misc_feature 1..58: note = Synthetic Sequence
  source 1..58: mol_type = other RNA

SEQ ID NO: 6 - RNA, 100 nt, synthetic construct
  misc_feature 1..100: note = Synthetic Sequence
  source 1..100: mol_type = other RNA
ctagttccagacacctcccaagcacgcagcaatgcagctcaaaacgcttagcctagccacacccccacgggaaacagcagtgattaacctttagcaataa

SEQ ID NO: 7 - DNA, 42 bp, synthetic construct
  misc_feature 1..42: note = Synthetic Sequence
  source 1..42: mol_type = other DNA
ttttttttttggtctcttttttttattgctaaaggttaatca

SEQ ID NO: 8 - DNA, 54 bp, synthetic construct
  misc_feature 1..54: note = Synthetic Sequence
  source 1..54: mol_type = other DNA
aggctaagcgttttgagctgcattgctgcgtgcttgggaggtgtctggaactag

SEQ ID NO: 9 - RNA, 120 nt, synthetic construct
  misc_feature 1..120: note = Synthetic Sequence
  source 1..120: mol_type = other RNA
tccaccagttttagagctagaaatagcaagttaaaataaggctagtccgttatcaacttgaaaaagtggcaccgagtcggtgcttttagatcggaagagcacacgtctgaactccagtca

SEQ ID NO: 10 - RNA, 162 nt, synthetic construct
  misc_feature 1..162: note = Synthetic Sequence
  source 1..162: mol_type = other RNA
ggtggaagctgtgttgccaagtttcagagctatgctggaaacagcatagcaagttgaaataaggctagtccgttatcaacttgaaaaagtggcaccgagtcggtgcagtctgtccagtcatttgtccattggcaacacgggcagggctgggagggttttttt

SEQ ID NO: 11 - DNA, 35 bp, synthetic construct
  misc_feature 1..35: note = Synthetic Sequence
  source 1..35: mol_type = other DNA
ttttttggtctctgactggagttcagacgtgtgct

SEQ ID NO: 12 - DNA, 44 bp, synthetic construct
  misc_feature 1..44: note = Synthetic Sequence
  source 1..44: mol_type = other DNA
tttttttttttttaaaaaaaccctcccagccctgcccgtgttgc